European Patent Specification EP 3 290 526 B1, published November 19, 2025. Title: Leaf mold resistance marker of Solanum Lycopersicum, leaf mold resistance Solanum Lycopersicum, production method of leaf mold resistance Solanum Lycopersicum and screening method of leaf mold resistance Solanum Lycopersicum. Applicant: Takii & Co.,Ltd. The sequence listing filed with the application follows.

SEQUENCE LISTING (18 sequences)

SEQ ID NO: 1 - DNA, 87 bp, Solanum Lycopersicum
tgatggaggaaacattacattctaatattttcgcagcaaacatctacactgtttgatgcttttaatgtatcagcctgttattcagaa

SEQ ID NO: 2 - DNA, 73 bp, Solanum Lycopersicum
ttttggttaagtgtggtgtcgcgaccaatttatgcacattttgattaatctactgagcacttgctacctacta

SEQ ID NO: 3 - DNA, 70 bp, Solanum Lycopersicum
tgggtgtcgtaaaagtctcataattgagatctcgcgtttgatatttgccattaaaatcgcgttgctaact

SEQ ID NO: 4 - DNA, 58 bp, Solanum Lycopersicum
tctaataccatctgcaagtttctgagcctcatctgacttcagcggacatctacttaag

SEQ ID NO: 5 - DNA, 80 bp, Solanum Lycopersicum
atagtgagtcaaacaattgtacattacatatcaatcactatgttatcacaacttccaactgattactagcttaagacatc

SEQ ID NO: 6 - DNA, 101 bp, Solanum Lycopersicum
gtgatggaggaaacattacattctaatattttcgcagcaaacatctacactgtttgatgcttttaatgtatcagcctgttattcagaagctgtcttcgttt

SEQ ID NO: 7 - DNA, 101 bp, Solanum Lycopersicum
tactcaaacttttttggttaagtgtggtgtcgcgaccaatttatgcacattttgattaatctactgagcacttgctacctactacctatatatgtattggg

SEQ ID NO: 8 - DNA, 101 bp, Solanum Lycopersicum
tcaagtttgacaatgtgtgggtgtcgtaaaagtctcataattgagatctcgcgtttgatatttgccattaaaatcgcgttgctaactcttgttttgttaat

SEQ ID NO: 9 - DNA, 101 bp, Solanum Lycopersicum
ctcgaaattgataagttttctctaataccatctgcaagtttctgagcctcatctgacttcagcggacatctacttaaggtctgtaaaacaatcaactttat

SEQ ID NO: 10 - DNA, 201 bp, Solanum Lycopersicum
gaaccaaatccattacgccaatgcgttcttattcttggcatttgaaaatctgaaaaatgagatagtgagtcaaacaactgtacattacatatcaatcactatgttatcacaacttccaactgattactagcttaagacatcagctaaggcttaatcttcagcttcttgaagttgttggaaagaaaaatatgcttcgtatcg

SEQ ID NO: 11 - DNA, 83 bp, Solanum Lycopersicum
gatgaactatggagaaatactgtagtgagtaaatatttgagaataagcagatagatgtaagataaaatgaatacatgacaaga

SEQ ID NO: 12 - DNA, 83 bp, Solanum Lycopersicum; identical to SEQ ID NO: 11

SEQ ID NO: 13 - DNA, 83 bp, Solanum Lycopersicum
tttcgtgtttcgtatttagaacttcttaatgaaaatcctggctcagcagctggtagttagtagagtgatttgtgggtgtatat

SEQ ID NO: 14 - DNA, 83 bp, Solanum Lycopersicum
tttcgtgtttcgtatttagaacttcttaatgaaaatcctggctccgccgctggtagttagtagagtgatttgtgggtgtatat

SEQ ID NO: 15 - DNA, 70 bp, Solanum Lycopersicum
tcacgagcagcaagaaagctattatcgctagtatccaatagtacgaaagagaacactccatccaacatgt

SEQ ID NO: 16 - DNA, 101 bp, Solanum Lycopersicum
tccaatggcatcacgagcagcaagaaagctattatcgcgagtatccaatagtacgaaagagaacactccatccaacatgtcaacaaaattttctccatact

SEQ ID NO: 17 - DNA, 81 bp, Solanum Lycopersicum
tacattctgttttatttgttccttacttgtcttagttgggctcatatctcattttgaatgtaaattacaggtgcaagacaa

SEQ ID NO: 18 - DNA, 81 bp, Solanum Lycopersicum; identical to SEQ ID NO: 17